European Patent Specification EP 3 596 130 B1, published December 4, 2024. Title: Dual-target fusion proteins comprising the Fc portion of an immunoglobulin. Applicant: SUNSHINE LAKE PHARMA CO., LTD. The sequence listing filed with the application follows.

SEQUENCE LISTING (31 sequences)

SEQ ID NO: 1 - protein, 31 aa, Artificial sequence
HGEGTFTSDVSSYLEEQAAKEFIAWLVKGGG

SEQ ID NO: 2 - protein, 228 aa, Artificial sequence
ESKYGPPCPPCPAPEAAGGPSVFLFPPKPKDTLMISRTPEVTCVVVDVSQEDPEVQFNWYVDGVEVHNAKTKPREEQFNSTYRVVSVLTVLHQDWLNGKEYKCKVSNKGLPSSIEKTISKAKGQPREPQVYTLPPSQEEMTKNQVSLTCLVKGFYPSDIAVEWESNGQPENNYKTTPPVLDSDGSFFLYSKLTVDKSRWQEGNVFSCSVMHEALHNHYTQKSLSLSLG

SEQ ID NO: 3 - protein, 275 aa, Artificial sequence
HGEGTFTSDVSSYLEEQAAKEFIAWLVKGGGGGGGSGGGGSGGGGSAESKYGPPCPPCPAPEAAGGPSVFLFPPKPKDTLMISRTPEVTCVVVDVSQEDPEVQFNWYVDGVEVHNAKTKPREEQFNSTYRVVSVLTVLHQDWLNGKEYKCKVSNKGLPSSIEKTISKAKGQPREPQVYTLPPSQEEMTKNQVSLTCLVKGFYPSDIAVEWESNGQPENNYKTTPPVLDSDGSFFLYSRLTVDKSRWQEGNVFSCSVMHEALHNHYTQKSLSLSLG

SEQ ID NO: 4 - protein, 424 aa, Artificial sequence
ESKYGPPCPPCPAPEAAGGPSVFLFPPKPKDTLMISRTPEVTCVVVDVSQEDPEVQFNWYVDGVEVHNAKTKPREEQFNSTYRVVSVLTVLHQDWLNGKEYKCKVSNKGLPSSIEKTISKAKGQPREPQVYTLPPSQEEMTKNQVSLTCLVKGFYPSDIAVEWESNGQPENNYKTTPPVLDSDGSFFLYSKLTVDKSRWQEGNVFSCSVMHEALHNHYTQKSLSLSLGGGGGSGGGGSGGGGSHPIPDSSPLLQFGGQVRQRYLYTDDAQQTEAHLEIREDGTVGGAADQSPESLLQLKALKPGVIQILGVKTSRFLCQRPDGALYGSLHFDPEACSFRERLLEDGYNVYQSEAHGLPLHLPGNKSPHRDPAPRGPARFLPLPGLPPALPEPPGILAPQPPDVGSSDPLSMVGGSQGRSPSYAS

SEQ ID NO: 5 - protein, 470 aa, Artificial sequence
HGEGTFTSDVSSYLEEQAAKEFIAWLVKGGGGGGGSGGGGSGGGGSESKYGPPCPPCPAPEAAGGPSVFLFPPKPKDTLMISRTPEVTCVVVDVSQEDPEVQFNWYVDGVEVHNAKTKPREEQFNSTYRVVSVLTVLHQDWLNGKEYKCKVSNKGLPSSIEKTISKAKGQPREPQVYTLPPSQEEMTKNQVSLTCLVKGFYPSDIAVEWESNGQPENNYKTTPPVLDSDGSFFLYSKLTVDKSRWQEGNVFSCSVMHEALHNHYTQKSLSLSLGGGGGSGGGGSGGGGSHPIPDSSPLLQFGGQVRQRYLYTDDAQQTEAHLEIREDGTVGGAADQSPESLLQLKALKPGVIQILGVKTSRFLCQRPDGALYGSLHFDPEACSFRERLLEDGYNVYQSEAHGLPLHLPGNKSPHRDPAPRGPARFLPLPGLPPALPEPPGILAPQPPDVGSSDPLSMVGGSQGRSPSYAS

SEQ ID NO: 6 - protein, 181 aa, Artificial sequence
HPIPDSSPLLQFGGQVRQRYLYTDDAQQTEAHLEIREDGTVGGAADQSPESLLQLKALKPGVIQILGVKTSRFLCQRPDGALYGSLHFDPEACSFRERLLEDGYNVYQSEAHGLPLHLPGNKSPHRDPAPRGPARFLPLPGLPPALPEPPGILAPQPPDVGSSDPLSMVGGSQGRSPSYAS

SEQ ID NO: 7 - protein, 31 aa, Artificial sequence
  misc_feature (2)..(2): Xaa at position 2 is Gly or Val
  misc_feature (16)..(16): Xaa at position 16 is Glu or Gly
  misc_feature (27)..(28): Xaa at position 27 is Val or Lys. Xaa at position 28 is Lys or Asn
  misc_feature (30)..(31): Xaa at position 30 is Gly or Glu. Xaa at position 31 is Gly or Pro
HXEGTFTSDVSSYLEXQAAKEFIAWLXXGXX

SEQ ID NO: 8 - protein, 229 aa, Artificial sequence
  misc_feature (15)..(17): Xaa at position 15 is Pro or Glu. Xaa at position 16 is Phe, Val or Ala. Xaa at position 17 is Leu, Glu or Ala
  misc_feature (79)..(79): Xaa at position 79 is Asn or Ala
  misc_feature (229)..(229): Xaa at position 229 is Lys or absent
ESKYGPPCPPCPAPXXXGGPSVFLFPPKPKDTLMISRTPEVTCVVVDVSQEDPEVQFNWYVDGVEVHNAKTKPREEQFXSTYRVVSVLTVLHQDWLNGKEYKCKVSNKGLPSSIEKTISKAKGQPREPQVYTLPPSQEEMTKNQVSLTCLVKGFYPSDIAVEWESNGQPENNYKTTPPVLDSDGSFFLYSKLTVDKSRWQEGNVFSCSVMHEALHNHYTQKSLSLSLGX

SEQ ID NO: 9 - protein, 181 aa, Artificial sequence
  misc_feature (45)..(45): Xaa at position 45 is selected from Ala, Lys, Arg, Glu or Gln
  misc_feature (98)..(98): Xaa at position 98 is selected from Leu, Asp, Arg, Glu, Gln, Lys or Thr
  misc_feature (100)..(100): Xaa at position 100 is selected from Leu or Lys
  misc_feature (118)..(118): Xaa at position 118 is selected from Leu or Cys
  misc_feature (134)..(134): Xaa at position 134 is selected from Ala or Cys
  misc_feature (150)..(152): Xaa at position 150 is selected from Pro or Ala. Xaa at position 151 is selected from Gly or Ala. Xaa at position 152 is selected from Ile or Val
  misc_feature (167)..(167): Xaa at position 167 is selected from Ser, His, Cys or Arg
  misc_feature (170)..(172): Xaa at position 170 is selected from Gly, Glu, Ala, Asp or Ser at position 170. Xaa at position 171 is selected from Pro, Ala, Glu, Gln, Trp, Cys, Gly or Thr; Met
  misc_feature (175)..(175): Xaa at position 175 is selected from Arg, Leu, His or Pro
  misc_feature (179)..(180): Xaa at position 179 is selected from Tyr, Ser, Ala or Phe. Xaa at position 180 is selected from Ala, Ser, Glu or Gly
HPIPDSSPLLQFGGQVRQRYLYTDDAQQTEAHLEIREDGTVGGAXDQSPESLLQLKALKPGVIQILGVKTSRFLCQRPDGALYGSLHFDPEACSFREXLXEDGYNVYQSEAHGLPLHXPGNKSPHRDPAPRGPXRFLPLPGLPPALPEPXXXLAPQPPDVGSSDPLXMVXXXQGXSPSXXS

SEQ ID NO: 10 - protein, 31 aa, Artificial sequence
  misc_feature (2)..(2): Xaa at position 2 is Gly or Val
  misc_feature (16)..(16): Xaa at position 16 is Glu or Gly
  misc_feature (30)..(30): Xaa at position 30 is Gly or GIu
HXEGTFTSDVSSYLEXQAAKEFIAWLVKGXG

SEQ ID NO: 11 - protein, 229 aa, Artificial sequence
  misc_feature (16)..(17): Xaa at position 16 is Phe, Val or Ala. and Xaa at position 17 is Leu, Glu or Ala
  misc_feature (229)..(229): Xaa at position 229 is Lys or absent
ESKYGPPCPPCPAPEXXGGPSVFLFPPKPKDTLMISRTPEVTCVVVDVSQEDPEVQFNWYVDGVEVHNAKTKPREEQFNSTYRVVSVLTVLHQDWLNGKEYKCKVSNKGLPSSIEKTISKAKGQPREPQVYTLPPSQEEMTKNQVSLTCLVKGFYPSDIAVEWESNGQPENNYKTTPPVLDSDGSFFLYSKLTVDKSRWQEGNVFSCSVMHEALHNHYTQKSLSLSLGX

SEQ ID NO: 12 - protein, 181 aa, Artificial sequence
  misc_feature (98)..(98): Xaa at position 98 is selected from Leu, Asp, Arg or Glu
  misc_feature (167)..(167): Xaa at position 167 is selected from Ser, His, Cys or Arg
  misc_feature (171)..(171): Xaa at position 171 is selected from Ala or Gly
  misc_feature (175)..(175): Xaa at position 175 is selected from Arg, Leu, or Pro
  misc_feature (179)..(179): The Xaa at position 179 is selected from Tyr, Ser or Phe
HPIPDSSPLLQFGGQVRQRYLYTDDAQQTEAHLEIREDGTVGGAVDQSPESLLQLKALKPGVIQILGVKTSRFLCQRPDGALYGSLHFDPEACSFREXLLEDGYNVYQSEAHGLPLHLPGNKSPHRDPAPRGPARFLPLPGLPPALPEPPGILAPQPPDVGSSDPLXMVGXSQGXSPSXAS

SEQ ID NO: 13 - protein, 15 aa, Artificial sequence
GGGGSGGGGSGGGGS

SEQ ID NO: 14 - protein, 31 aa, Artificial sequence
HAEGTFTSDVSSYLEGQAAKEFIAWLVKGRG

SEQ ID NO: 15 - protein, 181 aa, Artificial sequence
HPIPDSSPLLQFGGQVRQRYLYTDDAQQTEAHLEIREDGTVGGAADQSPESLLQLKALKPGVIQILGVKTSRFLCQRPDGALYGSLHFDPEACSFRELLLEDGYNVYQSEAHGLPLHLPGNKSPHRDPAPRGPARFLPLPGLPPALPEPPGILAPQPPDVGSSDPLSMVGPSQGRSPSYAS

SEQ ID NO: 16 - protein, 470 aa, Artificial sequence
HGEGTFTSDVSSYLEEQAAKEFIAWLVKGGGGGGGSGGGGSGGGGSESKYGPPCPPCPAPEAAGGPSVFLFPPKPKDTLMISRTPEVTCVVVDVSQEDPEVQFNWYVDGVEVHNAKTKPREEQFNSTYRVVSVLTVLHQDWLNGKEYKCKVSNKGLPSSIEKTISKAKGQPREPQVYTLPPSQEEMTKNQVSLTCLVKGFYPSDIAVEWESNGQPENNYKTTPPVLDSDGSFFLYSRLTVDKSRWQEGNVFSCSVMHEALHNHYTQKSLSLSLGGGGGSGGGGSGGGGSHPIPDSSPLLQFGGQVRQRYLYTDDAQQTEAHLEIREDGTVGGAADQSPESLLQLKALKPGVIQILGVKTSRFLCQRPDGALYGSLHFDPEACSFRERLLEDGYNVYQSEAHGLPLHLPGNKSPHRDPAPRGPARFLPLPGLPPALPEPPGILAPQPPDVGSSDPLSMVGGSQGRSPSYAS

SEQ ID NO: 17 - protein, 470 aa, Artificial sequence
HGEGTFTSDVSSYLEEQAAKEFIAWLVKGGGGGGGSGGGGSGGGGSESKYGPPCPPCPAPEAAGGPSVFLFPPKPKDTLMISRTPEVTCVVVDVSQEDPEVQFNWYVDGVEVHNAKTKPREEQFNSTYRVVSVLTVLHQDWLNGKEYKCKVSNKGLPSSIEKTISKAKGQPREPQVYTLPPSQEEMTKNQVSLTCLVKGFYPSDIAVEWESNGQPENNYKTTPPVLDSDGSFFLYSKLTVDKSRWQEGNVFSCSVMHEALHNHYTQKSLSLSLGGGGGSGGGGSGGGGSHPIPDSSPLLQFGGQVRQRYLYTDDAQQTEAHLEIREDGTVGGAADQSPESLLQLKALKPGVIQILGVKTSRFLCQRPDGALYGSLHFDPEACSFRERLLEDGYNVYQSEAHGLPLHLPGNKSPHRDPAPRGPARFLPLPGLPPALPEPPGILAPQPPDVGSSDPLSMVGGSQGRSPSFAS

SEQ ID NO: 18 - protein, 470 aa, Artificial sequence
HGEGTFTSDVSSYLEEQAAKEFIAWLVKGGGGGGGSGGGGSGGGGSESKYGPPCPPCPAPEAAGGPSVFLFPPKPKDTLMISRTPEVTCVVVDVSQEDPEVQFNWYVDGVEVHNAKTKPREEQFNSTYRVVSVLTVLHQDWLNGKEYKCKVSNKGLPSSIEKTISKAKGQPREPQVYTLPPSQEEMTKNQVSLTCLVKGFYPSDIAVEWESNGQPENNYKTTPPVLDSDGSFFLYSKLTVDKSRWQEGNVFSCSVMHEALHNHYTQKSLSLSLGGGGGSGGGGSGGGGSHPIPDSSPLLQFGGQVRQRYLYTDDAQQTEAHLEIREDGTVGGAADQSPESLLQLKALKPGVIQILGVKTSRFLCQRPDGALYGSLHFDPEACSFRERLLEDGYNVYQSEAHGLPLHLPGNKSPHRDPAPRGPARFLPLPGLPPALPEPPGILAPQPPDVGSSDPLSMVGASQGRSPSYAS

SEQ ID NO: 19 - protein, 470 aa, Artificial sequence
HGEGTFTSDVSSYLEEQAAKEFIAWLVKGGGGGGGSGGGGSGGGGSESKYGPPCPPCPAPEAAGGPSVFLFPPKPKDTLMISRTPEVTCVVVDVSQEDPEVQFNWYVDGVEVHNAKTKPREEQFNSTYRVVSVLTVLHQDWLNGKEYKCKVSNKGLPSSIEKTISKAKGQPREPQVYTLPPSQEEMTKNQVSLTCLVKGFYPSDIAVEWESNGQPENNYKTTPPVLDSDGSFFLYSKLTVDKSRWQEGNVFSCSVMHEALHNHYTQKSLSLSLGGGGGSGGGGSGGGGSHPIPDSSPLLQFGGQVRQRYLYTDDAQQTEAHLEIREDGTVGGAADQSPESLLQLKALKPGVIQILGVKTSRFLCQRPDGALYGSLHFDPEACSFRERLLEDGYNVYQSEAHGLPLHLPGNKSPHRDPAPRGPARFLPLPGLPPALPEPPGILAPQPPDVGSSDPLHMVGASQGRSPSYAS

SEQ ID NO: 20 - protein, 470 aa, Artificial sequence
HGEGTFTSDVSSYLEEQAAKEFIAWLVKGGGGGGGSGGGGSGGGGSESKYGPPCPPCPAPEAAGGPSVFLFPPKPKDTLMISRTPEVTCVVVDVSQEDPEVQFNWYVDGVEVHNAKTKPREEQFNSTYRVVSVLTVLHQDWLNGKEYKCKVSNKGLPSSIEKTISKAKGQPREPQVYTLPPSQEEMTKNQVSLTCLVKGFYPSDIAVEWESNGQPENNYKTTPPVLDSDGSFFLYSKLTVDKSRWQEGNVFSCSVMHEALHNHYTQKSLSLSLGGGGGSGGGGSGGGGSHPIPDSSPLLQFGGQVRQRYLYTDDAQQTEAHLEIREDGTVGGAADQSPESLLQLKALKPGVIQILGVKTSRFLCQRPDGALYGSLHFDPEACSFRERLLEDGYNVYQSEAHGLPLHLPGNKSPHRDPAPRGPARFLPLPGLPPALPEPPGILAPQPPDVGSSDPLHMVGASQGLSPSYAS

SEQ ID NO: 21 - protein, 470 aa, Artificial sequence
HGEGTFTSDVSSYLEEQAAKEFIAWLVKGGGGGGGSGGGGSGGGGSESKYGPPCPPCPAPEAAGGPSVFLFPPKPKDTLMISRTPEVTCVVVDVSQEDPEVQFNWYVDGVEVHNAKTKPREEQFNSTYRVVSVLTVLHQDWLNGKEYKCKVSNKGLPSSIEKTISKAKGQPREPQVYTLPPSQEEMTKNQVSLTCLVKGFYPSDIAVEWESNGQPENNYKTTPPVLDSDGSFFLYSKLTVDKSRWQEGNVFSCSVMHEALHNHYTQKSLSLSLGGGGGSGGGGSGGGGSHPIPDSSPLLQFGGQVRQRYLYTDDAQQTEAHLEIREDGTVGGAADQSPESLLQLKALKPGVIQILGVKTSRFLCQRPDGALYGSLHFDPEACSFRERLLEDGYNVYQSEAHGLPLHLPGNKSPHRDPAPRGPARFLPLPGLPPALPEPPGILAPQPPDVGSSDPLSMVEALQGRSPSYAS

SEQ ID NO: 22 - protein, 470 aa, Artificial sequence
HGEGTFTSDVSSYLEEQAAKEFIAWLVKGGGGGGGSGGGGSGGGGSESKYGPPCPPCPAPEAAGGPSVFLFPPKPKDTLMISRTPEVTCVVVDVSQEDPEVQFNWYVDGVEVHNAKTKPREEQFNSTYRVVSVLTVLHQDWLNGKEYKCKVSNKGLPSSIEKTISKAKGQPREPQVYTLPPSQEEMTKNQVSLTCLVKGFYPSDIAVEWESNGQPENNYKTTPPVLDSDGSFFLYSKLTVDKSRWQEGNVFSCSVMHEALHNHYTQKSLSLSLGGGGGSGGGGSGGGGSHPIPDSSPLLQFGGQVRQRYLYTDDAQQTEAHLEIREDGTVGGAADQSPESLLQLKALKPGVIQILGVKTSRFLCQRPDGALYGSLHFDPEACSFRELLLEDGYNVYQSEAHGLPLHLPGNKSPHRDPAPRGPARFLPLPGLPPALPEPPGILAPQPPDVGSSDPLSMVGPSQGRSPSYAS

SEQ ID NO: 23 - DNA, 1272 bp, Artificial sequence
  DNA-S1F1
gagtctaagtacggccctccctgccctccttgtcctgctcctgaagctgctggcggcccttccgtgttcctgttccccccaaagcccaaggacaccctgatgatctcccggacccccgaagtgacctgcgtggtggtggatgtgtcccaggaagatcccgaggtgcagttcaattggtacgtggacggcgtggaagtgcacaacgccaagaccaagcccagagaggaacagttcaactccacctaccgggtggtgtccgtgctgacagtgctgcaccaggactggctgaacggcaaagagtacaagtgcaaggtgtccaacaagggcctgcccagctccatcgaaaagaccatctccaaggccaagggccagccccgggaaccccaggtgtacacactgcctccaagccaggaagagatgaccaagaaccaggtgtccctgacctgtctcgtgaaaggcttctacccctccgatatcgccgtggaatgggagtccaacggccagcctgagaacaactacaagaccaccccccctgtgctggactccgacggctccttcttcctgtactccaagctgaccgtggacaagtccagatggcaggaaggcaacgtgttctcctgctccgtgatgcacgaggccctgcacaaccactacacccagaagtccctgtccctgtctctgggaggcggcggaggatctggcggaggtggaagcggaggcggtggatctcaccccatccccgacagcagccccctgctgcagttcggcggccaggtgaggcagaggtacctgtacaccgacgacgcccagcagaccgaggcccacctggagatcagggaggacggcaccgtgggcggcgccgccgaccagagccccgagagcctgctgcagctgaaggccctgaagcccggcgtgatccagatcctgggcgtgaagaccagcaggttcctgtgccagaggcccgacggcgccctgtacggcagcctgcacttcgaccccgaggcctgcagcttcagggagaggctgctggaggacggctacaacgtgtaccagagcgaggcccacggcctgcccctgcacctgcccggcaacaagagcccccacagggaccccgcccccaggggccccgccaggttcctgcccctgcccggcctgccccccgccctgcccgagccccccggcatcctggccccccagccccccgacgtgggcagcagcgaccccctgagcatggtgggaggatcccagggcaggagccccagctacgccagc

SEQ ID NO: 24 - DNA, 1410 bp, Artificial sequence
  DNA-D1F1
catggcgagggcacctttacctccgacgtgtcctcctacctggaagaacaggccgccaaagagtttatcgcctggctcgtgaagggcggtggtggcggcggaggatctggcggaggtggaagcggaggcggtggatctgagtctaagtacggccctccctgccctccttgtcctgctcctgaagctgctggcggcccttccgtgttcctgttccccccaaagcccaaggacaccctgatgatctcccggacccccgaagtgacctgcgtggtggtggatgtgtcccaggaagatcccgaggtgcagttcaattggtacgtggacggcgtggaagtgcacaacgccaagaccaagcccagagaggaacagttcaactccacctaccgggtggtgtccgtgctgacagtgctgcaccaggactggctgaacggcaaagagtacaagtgcaaggtgtccaacaagggcctgcccagctccatcgaaaagaccatctccaaggccaagggccagccccgggaaccccaggtgtacacactgcctccaagccaggaagagatgaccaagaaccaggtgtccctgacctgtctcgtgaaaggcttctacccctccgatatcgccgtggaatgggagtccaacggccagcctgagaacaactacaagaccaccccccctgtgctggactccgacggctccttcttcctgtactccaagctgaccgtggacaagtccagatggcaggaaggcaacgtgttctcctgctccgtgatgcacgaggccctgcacaaccactacacccagaagtccctgtccctgtctctgggaggcggcggaggatctggcggaggtggaagcggaggcggtggatctcaccccatccccgacagcagccccctgctgcagttcggcggccaggtgaggcagaggtacctgtacaccgacgacgcccagcagaccgaggcccacctggagatcagggaggacggcaccgtgggcggcgccgccgaccagagccccgagagcctgctgcagctgaaggccctgaagcccggcgtgatccagatcctgggcgtgaagaccagcaggttcctgtgccagaggcccgacggcgccctgtacggcagcctgcacttcgaccccgaggcctgcagcttcagggagaggctgctggaggacggctacaacgtgtaccagagcgaggcccacggcctgcccctgcacctgcccggcaacaagagcccccacagggaccccgcccccaggggccccgccaggttcctgcccctgcccggcctgccccccgccctgcccgagccccccggcatcctggccccccagccccccgacgtgggcagcagcgaccccctgagcatggtgggaggatcccagggcaggagccccagctacgccagc

SEQ ID NO: 25 - DNA, 1410 bp, Artificial sequence
  DNA-D1F2
catggcgagggcacctttacctccgacgtgtcctcctacctggaagaacaggccgccaaagagtttatcgcctggctcgtgaagggcggtggtggcggcggaggatctggcggaggtggaagcggaggcggtggatctgagtctaagtacggccctccctgccctccttgtcctgctcctgaagctgctggcggcccttccgtgttcctgttccccccaaagcccaaggacaccctgatgatctcccggacccccgaagtgacctgcgtggtggtggatgtgtcccaggaagatcccgaggtgcagttcaattggtacgtggacggcgtggaagtgcacaacgccaagaccaagcccagagaggaacagttcaactccacctaccgggtggtgtccgtgctgacagtgctgcaccaggactggctgaacggcaaagagtacaagtgcaaggtgtccaacaagggcctgcccagctccatcgaaaagaccatctccaaggccaagggccagccccgggaaccccaggtgtacacactgcctccaagccaggaagagatgaccaagaaccaggtgtccctgacctgtctcgtgaaaggcttctacccctccgatatcgccgtggaatgggagtccaacggccagcctgagaacaactacaagaccaccccccctgtgctggactccgacggctccttcttcctgtactccaggctgaccgtggacaagtccagatggcaggaaggcaacgtgttctcctgctccgtgatgcacgaggccctgcacaaccactacacccagaagtccctgtccctgtctctgggaggcggcggaggatctggcggaggtggaagcggaggcggtggatctcaccccatccccgacagcagccccctgctgcagttcggcggccaggtgaggcagaggtacctgtacaccgacgacgcccagcagaccgaggcccacctggagatcagggaggacggcaccgtgggcggcgccgccgaccagagccccgagagcctgctgcagctgaaggccctgaagcccggcgtgatccagatcctgggcgtgaagaccagcaggttcctgtgccagaggcccgacggcgccctgtacggcagcctgcacttcgaccccgaggcctgcagcttcagggagaggctgctggaggacggctacaacgtgtaccagagcgaggcccacggcctgcccctgcacctgcccggcaacaagagcccccacagggaccccgcccccaggggccccgccaggttcctgcccctgcccggcctgccccccgccctgcccgagccccccggcatcctggccccccagccccccgacgtgggcagcagcgaccccctgagcatggtgggaggatcccagggcaggagccccagctacgccagc

SEQ ID NO: 26 - DNA, 1410 bp, Artificial sequence
  DNA-D2F1
catggcgagggcacctttacctccgacgtgtcctcctacctggaagaacaggccgccaaagagtttatcgcctggctcgtgaagggcggtggtggcggcggaggatctggcggaggtggaagcggaggcggtggatctgagtctaagtacggccctccctgccctccttgtcctgctcctgaagctgctggcggcccttccgtgttcctgttccccccaaagcccaaggacaccctgatgatctcccggacccccgaagtgacctgcgtggtggtggatgtgtcccaggaagatcccgaggtgcagttcaattggtacgtggacggcgtggaagtgcacaacgccaagaccaagcccagagaggaacagttcaactccacctaccgggtggtgtccgtgctgacagtgctgcaccaggactggctgaacggcaaagagtacaagtgcaaggtgtccaacaagggcctgcccagctccatcgaaaagaccatctccaaggccaagggccagccccgggaaccccaggtgtacacactgcctccaagccaggaagagatgaccaagaaccaggtgtccctgacctgtctcgtgaaaggcttctacccctccgatatcgccgtggaatgggagtccaacggccagcctgagaacaactacaagaccaccccccctgtgctggactccgacggctccttcttcctgtactccaagctgaccgtggacaagtccagatggcaggaaggcaacgtgttctcctgctccgtgatgcacgaggccctgcacaaccactacacccagaagtccctgtccctgtctctgggaggcggcggaggatctggcggaggtggaagcggaggcggtggatctcaccccatccccgacagcagccccctgctgcagttcggcggccaggtgaggcagaggtacctgtacaccgacgacgcccagcagaccgaggcccacctggagatcagggaggacggcaccgtgggcggcgccgccgaccagagccccgagagcctgctgcagctgaaggccctgaagcccggcgtgatccagatcctgggcgtgaagaccagcaggttcctgtgccagaggcccgacggcgccctgtacggcagcctgcacttcgaccccgaggcctgcagcttcagggagaggctgctggaggacggctacaacgtgtaccagagcgaggcccacggcctgcccctgcacctgcccggcaacaagagcccccacagggaccccgcccccaggggccccgccaggttcctgcccctgcccggcctgccccccgccctgcccgagccccccggcatcctggccccccagccccccgacgtgggcagcagcgaccccctgagcatggtgggaggatcccagggcaggagccccagcttcgccagc

SEQ ID NO: 27 - DNA, 1410 bp, Artificial sequence
  DNA-D3F1
catggcgagggcacctttacctccgacgtgtcctcctacctggaagaacaggccgccaaagagtttatcgcctggctcgtgaagggcggtggtggcggcggaggatctggcggaggtggaagcggaggcggtggatctgagagcaagtacggccccccctgtcctccttgccccgcccctgaggccgccggcggccctagcgtgtttctgtttccccccaagcctaaagacaccctgatgatctccaggacccctgaggtgacctgtgtggtggtggacgtgagccaggaggaccccgaggtgcagttcaactggtacgtggatggcgtggaagtgcacaacgccaagaccaagcccagggaggagcaattcaacagcacctacagggtggtgagcgtcctcaccgtcctgcatcaggactggctgaacggcaaggagtacaagtgcaaagtgtccaacaagggcctgccttcctccatcgagaagaccatctccaaggctaagggccagcccagggaaccccaagtgtacaccctccccccctcccaggaggagatgaccaaaaaccaagtctccctgacctgcctggtgaagggcttctacccctccgatattgccgtcgagtgggagagcaacggccagcccgagaacaactataagaccaccccccccgtgctggattccgacggttcttttttcctgtatagcaagctgaccgtggacaagtccaggtggcaggagggcaacgtgttctcctgcagcgtgatgcacgaggccctccacaaccactacacccagaaatccctgtccctgtccctcggcggcggaggcggctccggcggcggcggcagcggaggcggaggaagccatcccattcccgactccagccccctgctgcagtttggcggccaagtgaggcagagatacctgtacaccgacgatgcccaacagacagaggctcacctggaaatcagggaggacggcaccgtgggcggagctgctgatcagagccccgagtccctcctccagctgaaggccctgaagcccggagtgatccagatcctgggcgtgaagacatccaggttcctgtgccagagacccgatggcgccctgtacggaagcctgcacttcgaccccgaggcttgctccttcagggagaggctgctggaggacggctacaacgtgtaccagtccgaggctcacggactccctctgcacctgcctggcaacaagagccctcacagagaccccgcccctagaggccctgctaggtttctgcccctgcctggcctgcctcctgctctgcccgagccccctggtattttagctcctcagcctcccgatgtgggaagcagcgaccccctgagcatggtgggagctagccagggcaggagccctagctacgccagc

SEQ ID NO: 28 - DNA, 1410 bp, Artificial sequence
  DNA-D4F1
catggcgagggcacctttacctccgacgtgtcctcctacctggaagaacaggccgccaaagagtttatcgcctggctcgtgaagggcggtggtggcggcggaggatctggcggaggtggaagcggaggcggtggatctgagagcaagtacggccccccctgtcctccttgccccgcccctgaggccgccggcggccctagcgtgtttctgtttccccccaagcctaaagacaccctgatgatctccaggacccctgaggtgacctgtgtggtggtggacgtgagccaggaggaccccgaggtgcagttcaactggtacgtggatggcgtggaagtgcacaacgccaagaccaagcccagggaggagcaattcaacagcacctacagggtggtgagcgtcctcaccgtcctgcatcaggactggctgaacggcaaggagtacaagtgcaaagtgtccaacaagggcctgccttcctccatcgagaagaccatctccaaggctaagggccagcccagggaaccccaagtgtacaccctccccccctcccaggaggagatgaccaaaaaccaagtctccctgacctgcctggtgaagggcttctacccctccgatattgccgtcgagtgggagagcaacggccagcccgagaacaactataagaccaccccccccgtgctggattccgacggttcttttttcctgtatagcaagctgaccgtggacaagtccaggtggcaggagggcaacgtgttctcctgcagcgtgatgcacgaggccctccacaaccactacacccagaaatccctgtccctgtccctcggcggcggaggcggctccggcggcggcggcagcggaggcggaggaagccatcccattcccgactccagccccctgctgcagtttggcggccaagtgaggcagagatacctgtacaccgacgatgcccaacagacagaggctcacctggaaatcagggaggacggcaccgtgggcggagctgctgatcagagccccgagtccctcctccagctgaaggccctgaagcccggagtgatccagatcctgggcgtgaagacatccaggttcctgtgccagagacccgatggcgccctgtacggaagcctgcacttcgaccccgaggcttgctccttcagggagaggctgctggaggacggctacaacgtgtaccagtccgaggctcacggactccctctgcacctgcctggcaacaagagccctcacagagaccccgcccctagaggccctgctaggtttctgcccctgcctggcctgcctcctgctctgcccgagccccctggtattttagctcctcagcctcccgatgtgggaagcagcgaccccctgcacatggtgggagctagccagggcaggagccctagctacgccagc

SEQ ID NO: 29 - DNA, 1410 bp, Artificial sequence
  DNA-D5F1
catggcgagggcacctttacctccgacgtgtcctcctacctggaagaacaggccgccaaagagtttatcgcctggctcgtgaagggcggtggtggcggcggaggatctggcggaggtggaagcggaggcggtggatctgagagcaagtacggccccccctgtcctccttgccccgcccctgaggccgccggcggccctagcgtgtttctgtttccccccaagcctaaagacaccctgatgatctccaggacccctgaggtgacctgtgtggtggtggacgtgagccaggaggaccccgaggtgcagttcaactggtacgtggatggcgtggaagtgcacaacgccaagaccaagcccagggaggagcaattcaacagcacctacagggtggtgagcgtcctcaccgtcctgcatcaggactggctgaacggcaaggagtacaagtgcaaagtgtccaacaagggcctgccttcctccatcgagaagaccatctccaaggctaagggccagcccagggaaccccaagtgtacaccctccccccctcccaggaggagatgaccaaaaaccaagtctccctgacctgcctggtgaagggcttctacccctccgatattgccgtcgagtgggagagcaacggccagcccgagaacaactataagaccaccccccccgtgctggattccgacggttcttttttcctgtatagcaagctgaccgtggacaagtccaggtggcaggagggcaacgtgttctcctgcagcgtgatgcacgaggccctccacaaccactacacccagaaatccctgtccctgtccctcggcggcggaggcggctccggcggcggcggcagcggaggcggaggaagccatcccattcccgactccagccccctgctgcagtttggcggccaagtgaggcagagatacctgtacaccgacgatgcccaacagacagaggctcacctggaaatcagggaggacggcaccgtgggcggagctgctgatcagagccccgagtccctcctccagctgaaggccctgaagcccggagtgatccagatcctgggcgtgaagacatccaggttcctgtgccagagacccgatggcgccctgtacggaagcctgcacttcgaccccgaggcttgctccttcagggagaggctgctggaggacggctacaacgtgtaccagtccgaggctcacggactccctctgcacctgcctggcaacaagagccctcacagagaccccgcccctagaggccctgctaggtttctgcccctgcctggcctgcctcctgctctgcccgagccccctggtattttagctcctcagcctcccgatgtgggaagcagcgaccccctgcacatggtgggagctagccagggcctgagccctagctacgccagc

SEQ ID NO: 30 - DNA, 1410 bp, Artificial sequence
  DNA-D6F1
catggcgagggcacctttacctccgacgtgtcctcctacctggaagaacaggccgccaaagagtttatcgcctggctcgtgaagggcggtggtggcggcggaggatctggcggaggtggaagcggaggcggtggatctgagtctaagtacggccctccctgccctccttgtcctgctcctgaagctgctggcggcccttccgtgttcctgttccccccaaagcccaaggacaccctgatgatctcccggacccccgaagtgacctgcgtggtggtggatgtgtcccaggaagatcccgaggtgcagttcaattggtacgtggacggcgtggaagtgcacaacgccaagaccaagcccagagaggaacagttcaactccacctaccgggtggtgtccgtgctgacagtgctgcaccaggactggctgaacggcaaagagtacaagtgcaaggtgtccaacaagggcctgcccagctccatcgaaaagaccatctccaaggccaagggccagccccgggaaccccaggtgtacacactgcctccaagccaggaagagatgaccaagaaccaggtgtccctgacctgtctcgtgaaaggcttctacccctccgatatcgccgtggaatgggagtccaacggccagcctgagaacaactacaagaccaccccccctgtgctggactccgacggctccttcttcctgtactccaagctgaccgtggacaagtccagatggcaggaaggcaacgtgttctcctgctccgtgatgcacgaggccctgcacaaccactacacccagaagtccctgtccctgtctctgggaggcggcggaggatctggcggaggtggaagcggaggcggtggatctcaccccatccccgacagcagccccctgctgcagttcggcggccaggtgaggcagaggtacctgtacaccgacgacgcccagcagaccgaggcccacctggagatcagggaggacggcaccgtgggcggcgccgccgaccagagccccgagagcctgctgcagctgaaggccctgaagcccggcgtgatccagatcctgggcgtgaagaccagcaggttcctgtgccagaggcccgacggcgccctgtacggcagcctgcacttcgaccccgaggcctgcagcttcagggagaggctgctggaggacggctacaacgtgtaccagagcgaggcccacggcctgcccctgcacctgcccggcaacaagagcccccacagggaccccgcccccaggggccccgccaggttcctgcccctgcccggcctgccccccgccctgcccgagccccccggcatcctggccccccagccccccgacgtgggcagcagcgaccccctgagcatggtggaggccctgcagggcaggagccccagctacgccagc

SEQ ID NO: 31 - DNA, 1410 bp, Artificial sequence
  DNA-D7F1
catggcgagggcacctttacctccgacgtgtcctcctacctggaagaacaggccgccaaagagtttatcgcctggctcgtgaagggcggtggtggcggcggaggatctggcggaggtggaagcggaggcggtggatctgagtctaagtacggccctccctgccctccttgtcctgctcctgaagctgctggcggcccttccgtgttcctgttccccccaaagcccaaggacaccctgatgatctcccggacccccgaagtgacctgcgtggtggtggatgtgtcccaggaagatcccgaggtgcagttcaattggtacgtggacggcgtggaagtgcacaacgccaagaccaagcccagagaggaacagttcaactccacctaccgggtggtgtccgtgctgacagtgctgcaccaggactggctgaacggcaaagagtacaagtgcaaggtgtccaacaagggcctgcccagctccatcgaaaagaccatctccaaggccaagggccagccccgggaaccccaggtgtacacactgcctccaagccaggaagagatgaccaagaaccaggtgtccctgacctgtctcgtgaaaggcttctacccctccgatatcgccgtggaatgggagtccaacggccagcctgagaacaactacaagaccaccccccctgtgctggactccgacggctccttcttcctgtactccaagctgaccgtggacaagtccagatggcaggaaggcaacgtgttctcctgctccgtgatgcacgaggccctgcacaaccactacacccagaagtccctgtccctgtctctgggaggcggcggaggatctggcggaggtggaagcggaggcggtggatctcaccccatccccgacagcagccccctgctgcagttcggcggccaggtgaggcagaggtacctgtacaccgacgacgcccagcagaccgaggcccacctggagatcagggaggacggcaccgtgggcggcgccgccgaccagagccccgagagcctgctgcagctgaaggccctgaagcccggcgtgatccagatcctgggcgtgaagaccagcaggttcctgtgccagaggcccgacggcgccctgtacggcagcctgcacttcgaccccgaggcctgcagcttcagggagctgctgctggaggacggctacaacgtgtaccagagcgaggcccacggcctgcccctgcacctgcccggcaacaagagcccccacagggaccccgcccccaggggccccgccaggttcctgcccctgcccggcctgccccccgccctgcccgagccccccggcatcctggccccccagccccccgacgtgggcagcagcgaccccctgagcatggtgggaccttcccagggcaggagccccagctacgccagc